European Patent Application EP 4 226 943 A1, published August 16, 2023. Title: Therapeutic medication for immune and inframmatory diseases. Applicant: KEIO UNIVERSITY TAKEDA PHARMACEUTICAL COMPANY LIMITED. The sequence listing filed with the application follows.

SEQUENCE LISTING (8 sequences)

SEQ ID NO: 1 - protein, 244 aa, Homo sapiens
MRWCLLLIWAQGLRQAPLASGMMTGTIETTGNISAEKGGSIILQCHLSSTTAQVTQVNWEQQDQLLAICNADLGWHISPSFKDRVAPGPGLGLTLQSLTVNDTGEYFCIYHTYPDGTYTGRIFLEVLESSVAEHGARFQIPLLGAMAATLVVICTAVIVVVALTRKKKALRIHSVEGDLRRKSAGQEEWSPSAPSPPGSCVQAEAAPAGLCGEQRGEDCAELHDYFNVLSYRSLGNCSFFTETG

SEQ ID NO: 2 - protein, 8 aa, Artificial Sequence
  amino acid of clone M1-8 H-CDR1 amino acid sequence
GFPFANHV

SEQ ID NO: 3 - protein, 8 aa, Artificial Sequence
  amino acid of clone M1-8 H-CDR2 amino acid sequence
IFPFNEIT

SEQ ID NO: 4 - protein, 10 aa, Artificial Sequence
  amino acid of clone M1-8 H-CDR3 amino acid sequence
AREQLGSFAY

SEQ ID NO: 5 - protein, 6 aa, Artificial Sequence
  amino acid of clone M1-8 L-CDR1 amino acid sequence
QNIRSN

SEQ ID NO: 6 - protein, 9 aa, Artificial Sequence
  amino acid of clone M1-8 L-CDR3 amino acid sequence
QHINNWPFT

SEQ ID NO: 7 - protein, 117 aa, Artificial Sequence
  amino acid of M1-8 heavy chain variable region
  MISC_FEATURE (26)..(33): CDR1
  MISC_FEATURE (51)..(58): CDR2
  MISC_FEATURE (97)..(106): CDR3
QVQLQQSGPELVKPGSSVKMSCKASGFPFANHVMHWVKQQPGQGLEWIGCIFPFNEITNYNEKFKVKATLTSDKSSSTAYMELSSLASEDSAVYYCAREQLGSFAYWGQGTLVTVSA

SEQ ID NO: 8 - protein, 107 aa, Artificial Sequence
  amino acid of M1-8 light chain variable region
  MISC_FEATURE (27)..(32): CDR1
  MISC_FEATURE (50)..(52): CDR2
  MISC_FEATURE (89)..(97): CDR3
DIVLTQSPATLSVTPGDSVSLSCRASQNIRSNLHWYQQKSHESPRLLIKYASQSISGIPSRFSGSGSGTDFTLSINSVETEDFGMYFCQHINNWPFTFGSGTKLEIK